European Patent Specification EP 4 114 443 B1, published January 21, 2026. Title: SYNERGISTIC AND TARGETING COMPOSITIONS FOR TREATMENT OF ARTERIAL AND VENOUS THROMBOSIS. Applicant: ASTRAZENECA AB. The sequence listing filed with the application follows.

SEQUENCE LISTING (22 sequences)

SEQ ID NO: 1 - DNA, 1317 bp, Artificial Sequence
  source: /note="Description of Artificial Sequence: Synthetic polynucleotide"
  CDS (1)..(1314)
gaggtcctccctccaggactgaagtatggtattgtgctggatgccgggtcttcagggacccgcgtctacgtgtatcaatggccagcagaaaaagagaataataccggagtggtcagtcaaaccttcaaatgtagtgtgaaaggctctggaatctccagctatggaaataacccccaagatgtccccagagcctttgaggagtgtatgcaaaaagtcaaggggcaggttccatcccacctccacggatccacccccattcacctgggagccacggctgggatgcgcttgctgaggttgcaaaatgaaacagcagctaatgaagtccttgaaagcatccaaagctacttcaagtcccagccctttgactttaggggtgctcaaatcatttctgggcaagaagaaggggtatatggatggattacagccaactatttaatgggaaatttcctggagaagaacctgtggcacatgtgggtgcacccgcatggagtggaaaccacgggtgccctggacttaggtggtgcctccacccaaatatccttcgtggcaggagagaagatggatctgaacaccagcgacatcatgcaggtgtccctgtatggctacgtatacacgctctacacacacagcttccagtgctatggccggaatgaggctgagaagaagtttctggcaatgctcctgcagaattctcctaccaaaaaccatctcaccaatccctgttaccctcgggattatagcatcagcttcaccatgggccatgtatttgatagcctgtgcactgtggaccagaggccagaaagttataaccccaatgatgtcatcacttttgaaggaactggggacccatctctgtgtaaggagaaggtggcttccatatttgacttcaaagcttgccatgatcaagaaacctgttcttttgatggggtttatcagccaaagattaaagggccatttgtggcttttgcaggattctactacacagccagtgctttaaatctttcaggtagcttttccctggacaccttcaactccagcacctggaatttctgctcacagaattggagtcagctcccactgctgctccccaaatttgatgaggtatatgcccgctcttactgcttctcagccaactacatctaccacttgtttgtgaacggttacaaattcacagaggagacttggccccaaatacactttgaaaaagaagtggggaatagcagcatagcctggtctcttggctacatgctcagcctgaccaaccagatcccagctgaaagccctctgatccgtctgcccatagaaccacctgtctga

SEQ ID NO: 2 - protein, 438 aa, Artificial Sequence
  source: /note="Description of Artificial Sequence: Synthetic polypeptide"
EVLPPGLKYGIVLDAGSSGTRVYVYQWPAEKENNTGVVSQTFKCSVKGSGISSYGNNPQDVPRAFEECMQKVKGQVPSHLHGSTPIHLGATAGMRLLRLQNETAANEVLESIQSYFKSQPFDFRGAQIISGQEEGVYGWITANYLMGNFLEKNLWHMWVHPHGVETTGALDLGGASTQISFVAGEKMDLNTSDIMQVSLYGYVYTLYTHSFQCYGRNEAEKKFLAMLLQNSPTKNHLTNPCYPRDYSISFTMGHVFDSLCTVDQRPESYNPNDVITFEGTGDPSLCKEKVASIFDFKACHDQETCSFDGVYQPKIKGPFVAFAGFYYTASALNLSGSFSLDTFNSSTWNFCSQNWSQLPLLLPKFDEVYARSYCFSANYIYHLFVNGYKFTEETWPQIHFEKEVGNSSIAWSLGYMLSLTNQIPAESPLIRLPIEPPV

SEQ ID NO: 3 - DNA, 2403 bp, Artificial Sequence
  source: /note="Description of Artificial Sequence: Synthetic polynucleotide"
  CDS (1)..(2400)
atggagacagacacactcctgctatgggtactgctgctctgggttccaggttccactggtgacgcgcccgaggtgctgcccccaggcctgaagtacgggatcgtcctggacgccggaagctccggtacccgggtctatgtgtaccagtggcccgccgaaaaggagaacaatacaggcgtggtgtcacaaaccttcaagtgttcagtcaaaggtagtggaatttcttcatatgggaacaatccccaggatgtgcctagggcatttgaggaatgtatgcagaaagtcaagggccaggtcccatctcatctgcatggttcaactcccatccatctgggtgccactgcaggaatgaggctgctgcggctgcagaatgaaaccgcagccaacgaggtcctggaatccattcaaagttacttcaagtcccaaccttttgacttccgaggcgctcaaattatcagtggtcaggaagagggagtctatggctggatcaccgcaaactacctgatgggtaattttctggagaagaacctgtggcatatgtgggtccatccccacggtgtcgaaacaactggagccctggatctgggcggtgccagtacacagatctcatttgtcgctggtgagaaaatggacctgaacaccagcgatatcatgcaagtctctctgtatggatacgtctatactctgtacacccactctttccaatgttacggtcgcaacgaagccgagaagaaattcctggctatgctgctgcaaaattctcctaccaagaatcatctgactaatccttgctatcccagggactacagtattagctttactatgggccacgtgttcgattccctgtgcacagtcgaccagcggcccgagtcttacaatcccaacgatgtgatcaccttcgagggcactggtgacccctcactgtgcaaggagaaagtcgcaagtatcttcgactttaaggcttgccacgatcaagaaacttgctcctttgatggcgtctatcaaccaaaaatcaagggcccatttgtcgccttcgccgggttctattataccgcatccgccctgaacctgtctggtagcttcagtctggacacttttaattcaagtacatggaacttctgctctcagaattggagtcaactgcccctgctgctgcccaaattcgatgaggtgtacgctaggagttattgtttctcagcaaactatatctaccatctgtttgtgaatggctacaaattcacagaggagacatggccacaaattcactttgagaaagaggtcggaaattcatctattgcatggagcctggggtacatgctgagcctgactaatcagattcccgctgaatcacccctgatccgactgcctattgaaccacccgtcggctcgacgagcggcgggtcgacaagtggtggatctactagtggctctggatccggaattgctcaagtgctgaggggaactgtgactgacttcccaggcttcgatgaaagggcagacgctgagactctgcgcaaagcaatgaagggtctgggtacagatgaagagagtattctgacactgctgactagtcgctccaacgcccaaagacaggagattagcgcagcattcaaaactctgttcggtagggatctgctggacgatctgaaatctgaactgaccgggaaattcgagaaactgatcgtggccctgatgaaaccaagtcggctgtatgatgcatacgaactgaagcacgctctgaagggagccggcactaatgagaaggtgctgacagaaattatcgcatctcgaacccccgaggaactgcgcgctatcaagcaagtgtatgaagaggaatatggttccagcctggaggacgatgtcgtcggggatacctcaggttattaccaacgcatgctggtggtgctgctgcaggccaacagggaccctgacgctggcatcgatgaagcccaggtggaacaagacgcccaggcactgttccaagcaggggagctgaagtgggggaccgacgaggaaaagtttatcaccatctttggaactcggagtgtgagccatctgcgcaaagtctttgacaagtatatgacaatttccggcttccaaatcgaggaaaccattgatcgagagactagcggcaatctggaacagctgctgctggctgtggtgaaatcaatcagatcaattcctgcatatctggcagagacactgtattacgcaatgaaaggagccggaaccgacgatcatactctgattagagtcatggtcagtcggtccgagatcgacctgtttaacattagaaaggagttccgcaagaattttgcaacttccctgtactcaatgatcaaaggcgatacctctggtgactacaagaaagctctgctgctgctgtgcggcgaggatgactaa

SEQ ID NO: 4 - protein, 800 aa, Artificial Sequence
  source: /note="Description of Artificial Sequence: Synthetic polypeptide"
METDTLLLWVLLLWVPGSTGDAPEVLPPGLKYGIVLDAGSSGTRVYVYQWPAEKENNTGVVSQTFKCSVKGSGISSYGNNPQDVPRAFEECMQKVKGQVPSHLHGSTPIHLGATAGMRLLRLQNETAANEVLESIQSYFKSQPFDFRGAQIISGQEEGVYGWITANYLMGNFLEKNLWHMWVHPHGVETTGALDLGGASTQISFVAGEKMDLNTSDIMQVSLYGYVYTLYTHSFQCYGRNEAEKKFLAMLLQNSPTKNHLTNPCYPRDYSISFTMGHVFDSLCTVDQRPESYNPNDVITFEGTGDPSLCKEKVASIFDFKACHDQETCSFDGVYQPKIKGPFVAFAGFYYTASALNLSGSFSLDTFNSSTWNFCSQNWSQLPLLLPKFDEVYARSYCFSANYIYHLFVNGYKFTEETWPQIHFEKEVGNSSIAWSLGYMLSLTNQIPAESPLIRLPIEPPVGSTSGGSTSGGSTSGSGSGIAQVLRGTVTDFPGFDERADAETLRKAMKGLGTDEESILTLLTSRSNAQRQEISAAFKTLFGRDLLDDLKSELTGKFEKLIVALMKPSRLYDAYELKHALKGAGTNEKVLTEIIASRTPEELRAIKQVYEEEYGSSLEDDVVGDTSGYYQRMLVVLLQANRDPDAGIDEAQVEQDAQALFQAGELKWGTDEEKFITIFGTRSVSHLRKVFDKYMTISGFQIEETIDRETSGNLEQLLLAVVKSIRSIPAYLAETLYYAMKGAGTDDHTLIRVMVSRSEIDLFNIRKEFRKNFATSLYSMIKGDTSGDYKKALLLLCGEDD

SEQ ID NO: 5 - DNA, 60 bp, Artificial Sequence
  source: /note="Description of Artificial Sequence: Synthetic oligonucleotide"
  CDS (1)..(60)
ggctcgacgagcggcgggtcgacaagtggtggatctactagtggctctggagccacaatt

SEQ ID NO: 6 - protein, 20 aa, Artificial Sequence
  source: /note="Description of Artificial Sequence: Synthetic peptide"
GSTSGGSTSGGSTSGSGATI

SEQ ID NO: 7 - DNA, 2400 bp, Artificial Sequence
  source: /note="Description of Artificial Sequence: Synthetic polynucleotide"
  CDS (1)..(2397)
atgatgtcctttgtctctctgctcctggttggcatcctattccatgccacccaggccgacgcgcccgaggtgctgcccccaggcctgaagtacgggatcgtcctggacgccggaagctccggtacccgggtctatgtgtaccagtggcccgccgaaaaggagaacaatacaggcgtggtgtcacaaaccttcaagtgttcagtcaaaggtagtggaatttcttcatatgggaacaatccccaggatgtgcctagggcatttgaggaatgtatgcagaaagtcaagggccaggtcccatctcatctgcatggttcaactcccatccatctgggtgccactgcaggaatgaggctgctgcggctgcagaatgaaaccgcagccaacgaggtcctggaatccattcaaagttacttcaagtcccaaccttttgacttccgaggcgctcaaattatcagtggtcaggaagagggagtctatggctggatcaccgcaaactacctgatgggtaattttctggagaagaacctgtggcatatgtgggtccatccccacggtgtcgaaacaactggagccctggatctgggcggtgccagtacacagatctcatttgtcgctggtgagaaaatggacctgaacaccagcgatatcatgcaagtctctctgtatggatacgtctatactctgtacacccactctttccaatgttacggtcgcaacgaagccgagaagaaattcctggctatgctgctgcaaaattctcctaccaagaatcatctgactaatccttgctatcccagggactacagtattagctttactatgggccacgtgttcgattccctgtgcacagtcgaccagcggcccgagtcttacaatcccaacgatgtgatcaccttcgagggcactggtgacccctcactgtgcaaggagaaagtcgcaagtatcttcgactttaaggcttgccacgatcaagaaacttgctcctttgatggcgtctatcaaccaaaaatcaagggcccatttgtcgccttcgccgggttctattataccgcatccgccctgaacctgtctggtagcttcagtctggacacttttaattcaagtacatggaacttctgctctcagaattggagtcaactgcccctgctgctgcccaaattcgatgaggtgtacgctaggagttattgtttctcagcaaactatatctaccatctgtttgtgaatggctacaaattcacagaggagacatggccacaaattcactttgagaaagaggtcggaaattcatctattgcatggagcctggggtacatgctgagcctgactaatcagattcccgctgaatcacccctgatccgactgcctattgaaccacccgtcggctcgacgagcggcgggtcgacaagtggtggatctactagtggctctggagccacaattgctcaagtgctgaggggaactgtgactgacttcccaggcttcgatgaaagggcagacgctgagactctgcgcaaagcaatgaagggtctgggtacagatgaagagagtattctgacactgctgactagtcgctccaacgcccaaagacaggagattagcgcagcattcaaaactctgttcggtagggatctgctggacgatctgaaatctgaactgaccgggaaattcgagaaactgatcgtggccctgatgaaaccaagtcggctgtatgatgcatacgaactgaagcacgctctgaagggagccggcactaatgagaaggtgctgacagaaattatcgcatctcgaacccccgaggaactgcgcgctatcaagcaagtgtatgaagaggaatatggttccagcctggaggacgatgtcgtcggggatacctcaggttattaccaacgcatgctggtggtgctgctgcaggccaacagggaccctgacgctggcatcgatgaagcccaggtggaacaagacgcccaggcactgttccaagcaggggagctgaagtgggggaccgacgaggaaaagtttatcaccatctttggaactcggagtgtgagccatctgcgcaaagtctttgacaagtatatgacaatttccggcttccaaatcgaggaaaccattgatcgagagactagcggcaatctggaacagctgctgctggctgtggtgaaatcaatcagatcaattcctgcatatctggcagagacactgtattacgcaatgaaaggagccggaaccgacgatcatactctgattagagtcatggtcagtcggtccgagatcgacctgtttaacattagaaaggagttccgcaagaattttgcaacttccctgtactcaatgatcaaaggcgatacctctggtgactacaagaaagctctgctgctgctgtgcggcgaggatgactaa

SEQ ID NO: 8 - protein, 799 aa, Artificial Sequence
  source: /note="Description of Artificial Sequence: Synthetic polypeptide"
MMSFVSLLLVGILFHATQADAPEVLPPGLKYGIVLDAGSSGTRVYVYQWPAEKENNTGVVSQTFKCSVKGSGISSYGNNPQDVPRAFEECMQKVKGQVPSHLHGSTPIHLGATAGMRLLRLQNETAANEVLESIQSYFKSQPFDFRGAQIISGQEEGVYGWITANYLMGNFLEKNLWHMWVHPHGVETTGALDLGGASTQISFVAGEKMDLNTSDIMQVSLYGYVYTLYTHSFQCYGRNEAEKKFLAMLLQNSPTKNHLTNPCYPRDYSISFTMGHVFDSLCTVDQRPESYNPNDVITFEGTGDPSLCKEKVASIFDFKACHDQETCSFDGVYQPKIKGPFVAFAGFYYTASALNLSGSFSLDTFNSSTWNFCSQNWSQLPLLLPKFDEVYARSYCFSANYIYHLFVNGYKFTEETWPQIHFEKEVGNSSIAWSLGYMLSLTNQIPAESPLIRLPIEPPVGSTSGGSTSGGSTSGSGATIAQVLRGTVTDFPGFDERADAETLRKAMKGLGTDEESILTLLTSRSNAQRQEISAAFKTLFGRDLLDDLKSELTGKFEKLIVALMKPSRLYDAYELKHALKGAGTNEKVLTEIIASRTPEELRAIKQVYEEEYGSSLEDDVVGDTSGYYQRMLVVLLQANRDPDAGIDEAQVEQDAQALFQAGELKWGTDEEKFITIFGTRSVSHLRKVFDKYMTISGFQIEETIDRETSGNLEQLLLAVVKSIRSIPAYLAETLYYAMKGAGTDDHTLIRVMVSRSEIDLFNIRKEFRKNFATSLYSMIKGDTSGDYKKALLLLCGEDD

SEQ ID NO: 9 - DNA, 2334 bp, Artificial Sequence
  source: /note="Description of Artificial Sequence: Synthetic polynucleotide"
  CDS (1)..(2331)
gaggtgctgcccccaggcctgaagtacgggatcgtcctggacgccggaagctccggtacccgggtctatgtgtaccagtggcccgccgaaaaggagaacaatacaggcgtggtgtcacaaaccttcaagtgttcagtcaaaggtagtggaatttcttcatatgggaacaatccccaggatgtgcctagggcatttgaggaatgtatgcagaaagtcaagggccaggtcccatctcatctgcatggttcaactcccatccatctgggtgccactgcaggaatgaggctgctgcggctgcagaatgaaaccgcagccaacgaggtcctggaatccattcaaagttacttcaagtcccaaccttttgacttccgaggcgctcaaattatcagtggtcaggaagagggagtctatggctggatcaccgcaaactacctgatgggtaattttctggagaagaacctgtggcatatgtgggtccatccccacggtgtcgaaacaactggagccctggatctgggcggtgccagtacacagatctcatttgtcgctggtgagaaaatggacctgaacaccagcgatatcatgcaagtctctctgtatggatacgtctatactctgtacacccactctttccaatgttacggtcgcaacgaagccgagaagaaattcctggctatgctgctgcaaaattctcctaccaagaatcatctgactaatccttgctatcccagggactacagtattagctttactatgggccacgtgttcgattccctgtgcacagtcgaccagcggcccgagtcttacaatcccaacgatgtgatcaccttcgagggcactggtgacccctcactgtgcaaggagaaagtcgcaagtatcttcgactttaaggcttgccacgatcaagaaacttgctcctttgatggcgtctatcaaccaaaaatcaagggcccatttgtcgccttcgccgggttctattataccgcatccgccctgaacctgtctggtagcttcagtctggacacttttaattcaagtacatggaacttctgctctcagaattggagtcaactgcccctgctgctgcccaaattcgatgaggtgtacgctaggagttattgtttctcagcaaactatatctaccatctgtttgtgaatggctacaaattcacagaggagacatggccacaaattcactttgagaaagaggtcggaaattcatctattgcatggagcctggggtacatgctgagcctgactaatcagattcccgctgaatcacccctgatccgactgcctattgaaccacccgtcggctcgacgagcggcgggtcgacaagtggtggatctactagtggctctggagccacaattgctcaagtgctgaggggaactgtgactgacttcccaggcttcgatgaaagggcagacgctgagactctgcgcaaagcaatgaagggtctgggtacagatgaagagagtattctgacactgctgactagtcgctccaacgcccaaagacaggagattagcgcagcattcaaaactctgttcggtagggatctgctggacgatctgaaatctgaactgaccgggaaattcgagaaactgatcgtggccctgatgaaaccaagtcggctgtatgatgcatacgaactgaagcacgctctgaagggagccggcactaatgagaaggtgctgacagaaattatcgcatctcgaacccccgaggaactgcgcgctatcaagcaagtgtatgaagaggaatatggttccagcctggaggacgatgtcgtcggggatacctcaggttattaccaacgcatgctggtggtgctgctgcaggccaacagggaccctgacgctggcatcgatgaagcccaggtggaacaagacgcccaggcactgttccaagcaggggagctgaagtgggggaccgacgaggaaaagtttatcaccatctttggaactcggagtgtgagccatctgcgcaaagtctttgacaagtatatgacaatttccggcttccaaatcgaggaaaccattgatcgagagactagcggcaatctggaacagctgctgctggctgtggtgaaatcaatcagatcaattcctgcatatctggcagagacactgtattacgcaatgaaaggagccggaaccgacgatcatactctgattagagtcatggtcagtcggtccgagatcgacctgtttaacattagaaaggagttccgcaagaattttgcaacttccctgtactcaatgatcaaaggcgatacctctggtgactacaagaaagctctgctgctgctgtgcggcgaggatgactaa

SEQ ID NO: 10 - protein, 777 aa, Artificial Sequence
  source: /note="Description of Artificial Sequence: Synthetic polypeptide"
EVLPPGLKYGIVLDAGSSGTRVYVYQWPAEKENNTGVVSQTFKCSVKGSGISSYGNNPQDVPRAFEECMQKVKGQVPSHLHGSTPIHLGATAGMRLLRLQNETAANEVLESIQSYFKSQPFDFRGAQIISGQEEGVYGWITANYLMGNFLEKNLWHMWVHPHGVETTGALDLGGASTQISFVAGEKMDLNTSDIMQVSLYGYVYTLYTHSFQCYGRNEAEKKFLAMLLQNSPTKNHLTNPCYPRDYSISFTMGHVFDSLCTVDQRPESYNPNDVITFEGTGDPSLCKEKVASIFDFKACHDQETCSFDGVYQPKIKGPFVAFAGFYYTASALNLSGSFSLDTFNSSTWNFCSQNWSQLPLLLPKFDEVYARSYCFSANYIYHLFVNGYKFTEETWPQIHFEKEVGNSSIAWSLGYMLSLTNQIPAESPLIRLPIEPPVGSTSGGSTSGGSTSGSGATIAQVLRGTVTDFPGFDERADAETLRKAMKGLGTDEESILTLLTSRSNAQRQEISAAFKTLFGRDLLDDLKSELTGKFEKLIVALMKPSRLYDAYELKHALKGAGTNEKVLTEIIASRTPEELRAIKQVYEEEYGSSLEDDVVGDTSGYYQRMLVVLLQANRDPDAGIDEAQVEQDAQALFQAGELKWGTDEEKFITIFGTRSVSHLRKVFDKYMTISGFQIEETIDRETSGNLEQLLLAVVKSIRSIPAYLAETLYYAMKGAGTDDHTLIRVMVSRSEIDLFNIRKEFRKNFATSLYSMIKGDTSGDYKKALLLLCGEDD

SEQ ID NO: 11 - DNA, 63 bp, Artificial Sequence
  source: /note="Description of Artificial Sequence: Synthetic oligonucleotide"
  CDS (1)..(63)
ggctcgacgagcggcgggtcgacaagtggtggatctactagtggctctggatccggaattgct

SEQ ID NO: 12 - protein, 21 aa, Artificial Sequence
  source: /note="Description of Artificial Sequence: Synthetic peptide"
GSTSGGSTSGGSTSGSGSGIA

SEQ ID NO: 13 - DNA, 63 bp, Artificial Sequence
  source: /note="Description of Artificial Sequence: Synthetic oligonucleotide"
  CDS (1)..(63)
ggctcgacgagcggcgggtcgacaagtggtggatctactagtggctctggatccacaattgct

SEQ ID NO: 14 - protein, 21 aa, Artificial Sequence
  source: /note="Description of Artificial Sequence: Synthetic peptide"
GSTSGGSTSGGSTSGSGSTIA

SEQ ID NO: 15 - DNA, 63 bp, Artificial Sequence
  source: /note="Description of Artificial Sequence: Synthetic oligonucleotide"
  CDS (1)..(63)
ggctcgacgagcggcgggtcgacaagtggtggatctactagtggctctggagccacaattgct

SEQ ID NO: 16 - protein, 21 aa, Artificial Sequence
  source: /note="Description of Artificial Sequence: Synthetic peptide"
GSTSGGSTSGGSTSGSGATIA

SEQ ID NO: 17 - DNA, 63 bp, Artificial Sequence
  source: /note="Description of Artificial Sequence: Synthetic oligonucleotide"
  CDS (1)..(63)
ggctcgacgagcggcgggtcgacaagtggtggatctactagtggctctggacagacaattgct

SEQ ID NO: 18 - protein, 21 aa, Artificial Sequence
  source: /note="Description of Artificial Sequence: Synthetic peptide"
GSTSGGSTSGGSTSGSGQTIA

SEQ ID NO: 19 - protein, 5 aa, Artificial Sequence
  source: /note="Description of Artificial Sequence: Synthetic peptide"
GSTSG

SEQ ID NO: 20 - protein, 10 aa, Artificial Sequence
  source: /note="Description of Artificial Sequence: Synthetic peptide"
GSTSGGSTSG

SEQ ID NO: 21 - protein, 15 aa, Artificial Sequence
  source: /note="Description of Artificial Sequence: Synthetic peptide"
GSTSGGSTSGGSTSG

SEQ ID NO: 22 - protein, 9 aa, Artificial Sequence
  source: /note="Description of Artificial Sequence: Synthetic peptide"
PAPAPAPAP